European Patent Application EP 4 130 275 A1, published February 8, 2023. Title: Primer set and probe for detection of Staphylococcus argenteus. Applicant: Denka Company Limited Toho University. The sequence listing filed with the application follows.

SEQUENCE LISTING (15 sequences)

SEQ ID NO: 1 - DNA, 687 bp, Staphylococcus aureus strain NCTC13626
ttattgacctgaatcagcgttgtcttcgctccaaatatttaatttctctttttttgcttgtgcttcactttttcttaaaagttgttcatgtgtattgttaggtttataaacataagcaactttagccaagccttgacgaactaaagcttcgtttaccatttttccatcagcataaatatacgctaagccacgtccatatttatcagttctttgacctttgtcaaactcgacttcaattttctttgcattttctaccatttttttcgtaaatgcacttgcttcaggaccatatttctctacaccttttttaggatgctttgtttcaggtgtatcaaccaataatagtctgaatgtcattggttgacctttgtacattaatttaaccgtatcaccatcaatcgctttaattaatgtcgcaggttctttatgtaattttttagttgaagttgcactatatactgttggatcttcagaaccacttctatttacgccattatctgtttgtgatgcatttgctgagctacttagacttgaaactacaactaaagttaacactaaacaactagtagcgaaatagaaaaacctctttgcgtattgccctttcgaaacattactgatagccatccctataagtaatattgaaacgattgccatacatatgccagcacttaataagtattctgtcat

SEQ ID NO: 2 - DNA, 687 bp, Staphylococcus aureus strain AR221; identical to SEQ ID NO: 1

SEQ ID NO: 3 - DNA, 669 bp, Staphylococcus argenteus strain NCTC13711
ttattctgcgttaccttcactccaaatatttaaatgttctttttttgcttgtgcttcactttttcttaatagttgttcatgtgtgttattaggtttataaacatacgcaacttttgctagaccttgacgcactaaagcttggttaaccatcttaccatcagcatagatataagctaagccacgtccatatttatctgtcttttgacctttgtcaaattccacttctattttcttagcattctctaccatattcttcgtaaatgcacttgcttctgggccatatttttcaacgccttttttaggatgtttcgtttcaggcgtatcaattaataacaatctaaatgtcattggctttcctttatacattaacttaaccgtatcaccatcgatcgctttaattaatgtcgcaggttctttatgtaatttagtcgttgctgatttactgtattcagttgcattgctatttccctcttcatcagttagttgggatgctcctgcagattgattaaaattagaaactacaactaatgttaacactaagcaactaatagagaaaaataaaaatcttttcgctgtttgctttttagaaaatttacttatagccatcactacaagtactaatgaaacaattgtcgtaaatatgccagcacttaaaaagtattctgtcat

SEQ ID NO: 4 - DNA, 669 bp, Staphylococcus argenteus strain XNO106
ttattctgcgttaccttcactccaaatatttaaatgttcttttttcgcttgtgcttcactttttcttaatagttgttcatgtgtgttattaggtttataaacatacgcaacttttgctagaccttgacgcactaaagcttggttaaccatcttaccatcagcatagatataagctaagccacgtccatatttatctgtcttttgacctttgtcaaattccacttctattttcttagcattctctaccatattcttcgtaaatgcacttgcttctgggccatatttttcaacgccttttttaggatgtttcgtttcaggcgtatcaattaataacaatctaaatgtcattgcctttcctttatacattaacttaaccgtatcaccatcgatcgctttaattaatgtcgcaggttctttatgtaatttagtcgttgctgatttactgtattcagttgcattgctatttccctcttcatcagttagttgggatgctcctgcagattgattaaaattagaaactacaactaatgttaacactaagcaactaatagagaaaaataaaaatcttttcgctgtttgccttttagaaaatttacttatagccatcactacaagtactaatgaaacaattgccgtaaatatgccagcacttaaaaagtattctgtcat

SEQ ID NO: 5 - DNA, 669 bp, Staphylococcus schweitzeri strain FSCB5
ttattctgcgttaccttcactccaaatatttagatgttcttttttcgcttgtgcttcacttttccttaatagttgttcatgtgtattattaggtttatatacatatgcaacttttgctaatccttgacgtactaacgcttgattaaccattttgccatctgcataaatataagctaatccacgtccatatttatcagttttttgtcctttgtcaaattcaacttcaattttcttagcattctctaccatttttttcgtaaacgcgcttgcttctggtccgtatttttcaacgccttttttaggatgtttcgtttcgggcgtatcaattaataacaatctaaatgtcattggttgtcctttgtacattaacttaacagtatcaccatcaattgctttgattaatgtcgcaggctctttatgtaatttagtcgttactgatttgctatattcagttgcattgctatttccatcttcatcagttaattgggaagctccagcagtttgattaaaattagaaattacaactaatgttaacactacgcaactagtagagaaaaataaaaatcttttcgcggtttgcctttgagaaagtttacttatagccatcactataagtactaatgaaacaattgccgtaaatatgccagcacttaaaaagtattctgtcat

SEQ ID NO: 6 - DNA, 21 bp, Artificial Sequence
  Primer for Staphylococcus aureus
gtagcgaaawagaaaaacctc

SEQ ID NO: 7 - DNA, 24 bp, Artificial Sequence
  Primer for Staphylococcus aureus
atacttattaagtgctggcatatg

SEQ ID NO: 8 - DNA, 21 bp, Artificial Sequence
  Probe for Staphylococcus aureus
ccctataagtaatattgaaac

SEQ ID NO: 9 - DNA, 25 bp, Artificial Sequence
  Primer for Staphylococcus argenteus
ttccacttctattttcttagcattc

SEQ ID NO: 10 - DNA, 22 bp, Artificial Sequence
  Primer for Staphylococcus argenteus or schweitzeri
attaattgatacgccygaaacg

SEQ ID NO: 11 - DNA, 25 bp, Artificial Sequence
  Primer for Staphylococcus schweitzeri
ttcaacttcaattttyttagcattc

SEQ ID NO: 12 - DNA, 17 bp, Artificial Sequence
  Probe for Staphylococcus argenteus or schweitzeri
catatttttcaacgcct

SEQ ID NO: 13 - DNA, 23 bp, Artificial Sequence
  Prior Art Primer
gaaacaaagcatcctaaaaaagg

SEQ ID NO: 14 - DNA, 20 bp, Artificial Sequence
  Prior Art Primer
aagccttgacgaactaaagc

SEQ ID NO: 15 - DNA, 18 bp, Artificial Sequence
  Prior Art Probe
ataagctaagccacgtcc